European Patent Specification EP 4 063 498 B1, published April 24, 2024. Title: OXA-23-TYPE CARBAPENEMASE-RESISTANT HYBRIDOMA CELL LINE, AND MONOCLONAL ANTIBODY (mAb) AND USE THEREOF. Applicant: TIANJIN ERA BIOLOGY TECHNOLOGY CO., LTD. BEIJING GOLD MOUNTAINRIVER TECH DEVELOPMENT CO., LTD. The sequence listing filed with the application follows.

SEQUENCE LISTING (24 sequences)

SEQ ID NO: 1 - protein, 11 aa, Artificial Sequence
  The sequence is synthetized.
KASQDVSIAVA

SEQ ID NO: 2 - protein, 7 aa, Artificial Sequence
  The sequence is synthetized.
WASTRHT

SEQ ID NO: 3 - protein, 9 aa, Artificial Sequence
  The sequence is synthetized.
QQHYSTPYL

SEQ ID NO: 4 - protein, 10 aa, Artificial Sequence
  The sequence is synthetized.
GYTFTSYWMY

SEQ ID NO: 5 - protein, 17 aa, Artificial Sequence
  The sequence is synthetized.
EIYPTNGRTNYNEKFKT

SEQ ID NO: 6 - protein, 10 aa, Artificial Sequence
  The sequence is synthetized.
YYYGSYAMDY

SEQ ID NO: 7 - protein, 109 aa, Artificial Sequence
  The sequence is synthetized.
DIVMTQSHKFMSTSVGDRVSITCKASQDVSIAVAWFQQKPGQSPKLLIYWASTRHTGVPDRFTGSGSGTDYTLTISSVQAEDLALYYCQQHYSTPYLFGGGTKLEIKRA

SEQ ID NO: 8 - DNA, 327 bp, Artificial Sequence
  The sequence is synthetized.
gacattgtgatgacccagtctcacaaattcatgtccacatcagtaggagacagggtcagcatcacctgcaaggccagtcaggatgtgagtattgctgtagcctggtttcaacaaaaaccagggcaatctcctaaactactgatttactgggcatccacccggcacactggagtccctgatcgcttcacaggcagtggatctgggacagattatactctcaccatcagcagtgtgcaggctgaagacctggcactttattactgtcagcaacattatagcactccgtatttgttcggaggggggaccaagctggaaataaaacgggct

SEQ ID NO: 9 - protein, 118 aa, Artificial Sequence
  The sequence is synthetized.
VQLQQSGAELVKPGASVKLSCKTSGYTFTSYWMYWVKQRPGQGLEWIGEIYPTNGRTNYNEKFKTKATLTVDKSSSTAYMQLSSLTSEDSAVYYCAIYYYGSYAMDYWGQGTSVTVSS

SEQ ID NO: 10 - DNA, 354 bp, Artificial Sequence
  The sequence is synthetized.
gtgcagcttcagcagtcaggggctgaactggtgaagcctggggcctcagtgaagctgtcctgcaagacttctggctacaccttcaccagctactggatgtactgggtgaagcagaggcctggacaaggccttgagtggattggagagatttatcctaccaacggtcgtactaactacaatgagaaattcaagaccaaggccacactgactgtggacaaatcctccagcacagcctacatgcaactcagcagcctgacatctgaggactctgcggtctattactgtgcaatttattactacggtagctatgctatggactactggggtcaaggaacctcagtcaccgtctcctca

SEQ ID NO: 11 - protein, 11 aa, Artificial Sequence
  The sequence is synthetized.
KGSQDVRTAVA

SEQ ID NO: 12 - protein, 7 aa, Artificial Sequence
  The sequence is synthetized.
WASTRHT

SEQ ID NO: 13 - protein, 9 aa, Artificial Sequence
  The sequence is synthetized.
QQHYSIPYT

SEQ ID NO: 14 - protein, 10 aa, Artificial Sequence
  The sequence is synthetized.
GFSLTSYGVH

SEQ ID NO: 15 - protein, 19 aa, Artificial Sequence
  The sequence is synthetized.
VIWRGGNTDYNAAFMSRLS

SEQ ID NO: 16 - protein, 9 aa, Artificial Sequence
  The sequence is synthetized.
SLTTSTFDY

SEQ ID NO: 17 - protein, 109 aa, Artificial Sequence
  The sequence is synthetized.
DIVMTQSHKLMSTSVGDRVSITCKGSQDVRTAVAWYQQKPGQSPNLLIYWASTRHTGVPDRFTGSGSGTDYILTITSVQAEDLALYYCQQHYSIPYTFGGGTKLEIKRA

SEQ ID NO: 18 - DNA, 327 bp, Artificial Sequence
  The sequence is synthetized.
gacattgtgatgacccagtctcacaaactcatgtccacatcagtaggagacagggtcagcatcacctgcaagggcagtcaggatgtgaggactgctgtagcctggtatcaacaaaaaccaggacaatctcctaacctactgatttactgggcatccacccggcacactggagtccctgatcgcttcacaggcagtggatctgggacagattacattctcaccatcactagtgtgcaggctgaagacctggcactttattactgtcagcaacattatagtattccttacacgttcggaggggggaccaagctggaaataaaacgggct

SEQ ID NO: 19 - protein, 116 aa, Artificial Sequence
  The sequence is synthetized.
VQLKQSGPGLVQPSQSLSITCTVSGFSLTSYGVHWVRRSPGKGLEWLGVIWRGGNTDYNAAFMSRLSITKDNSKSQVFFKMTSLQGDDTAIYSCVKSLTTSTFDYWGQGTLVTVSS

SEQ ID NO: 20 - DNA, 348 bp, Artificial Sequence
  The sequence is synthetized.
gtgcaactgaagcagtcaggacctggcctagtgcagccctcacagagtctgtccataacctgcacagtctctggtttctcattaactagctatggtgtacactgggttcgccggtctccaggaaagggtctggagtggctgggagtgatctggagaggtggaaacacagactacaatgcagctttcatgtccagactgagcatcaccaaggacaactccaagagccaagttttctttaaaatgaccagtctgcaaggtgatgacaccgccatatactcctgtgtcaaatcccttactacgtctacgtttgattactggggccaagggactctggtcaccgtctcctca

SEQ ID NO: 21 - DNA, 23 bp, Artificial Sequence
  Upstream primer for a heavy chain framework region
saggtgmagctkcassartcwgg

SEQ ID NO: 22 - DNA, 32 bp, Artificial Sequence
  Downstream primer for a heavy chain variable region
tggggstgtygttttggctgmrgagacrgtga

SEQ ID NO: 23 - DNA, 26 bp, Artificial Sequence
  Upstream primer for a light chain leader peptide
atggattttcaagtgcagattttcag

SEQ ID NO: 24 - DNA, 30 bp, Artificial Sequence
  Downstream primer for a light chain variable region
ggatacagttggtgcagcatcagcccgttt